European Patent Application EP 4 806 921 A1, published September 16, 2026. Title: 항 CEACAM5 항체 및 이의 용도. Applicant: DAAN BIOTHERAPEUTICS CO., LTD. The sequence listing filed with the application follows.

SEQUENCE LISTING (48 sequences)

SEQ ID NO: 1 - protein, 5 aa, unidentified
NFGMN

SEQ ID NO: 2 - protein, 17 aa, unidentified
WINTYTGKPTYDDDFKG

SEQ ID NO: 3 - protein, 10 aa, unidentified
EAGKDYAMDY

SEQ ID NO: 4 - protein, 10 aa, unidentified
SASSSVTFMH

SEQ ID NO: 5 - protein, 7 aa, unidentified
DTSKLAS

SEQ ID NO: 6 - protein, 9 aa, unidentified
QQWNNYPWT

SEQ ID NO: 7 - protein, 119 aa, unidentified
QIQLVQSGSELKKPGASVKVSCKASGYTFTNFGMNWVRQAPGQGLEWMGWINTYTGKPTYDDDFKGRFVFSLDTSVSTAYLQISSLKAEDTAVYYCAREAGKDYAMDYWGQGTLVTVSS

SEQ ID NO: 8 - protein, 106 aa, unidentified
EIVLTQSPATLSLSPGERATLSCSASSSVTFMHWYQQKPGQAPRRLIYDTSKLASGIPARFSGSGSGTDYTLTISSLEPEDAAVYYCQQWNNYPWTFGGGTKVEIK

SEQ ID NO: 9 - protein, 106 aa, unidentified
DIQLTQSPSTLSASVGDRVTITCSASSSVTFMHWYQQKPGKAPKRLIYDTSKLASGVPSRFSGSGSGTEYTLTISSLQPDDAATYYCQQWNNYPWTFGGGTKVEIK

SEQ ID NO: 10 - protein, 106 aa, unidentified
EIVLTQSPATLSVSPGERATLSCSASSSVTFMHWYQQKPGQAPRRLIYDTSKLASGIPARFSGSGSGTEYTLTISSMQSEDAAVYYCQQWNNYPWTFGGGTKVEIK

SEQ ID NO: 11 - protein, 119 aa, unidentified
QIQLVQSGAEVKKPGASVKVSCKASGYTFTNFGMNWVRQAPGQGLEWMGWINTYTGKPTYDDDFKGRVTMTLDTSTSTAYMELRSLRSDDMAVYYCAREAGKDYAMDYWGQGTLVTVSS

SEQ ID NO: 12 - protein, 106 aa, unidentified
DIQLTQSPSSLSASVGDRVTITCSASSSVTFMHWYQQKPGKAPKRLIYDTSKLASGVPSRFSGSGSGTDYTLTISSLQPEDAATYYCQQWNNYPWTFGGGTKVEIK

SEQ ID NO: 13 - protein, 5 aa, unidentified
NYGVH

SEQ ID NO: 14 - protein, 16 aa, unidentified
LIWAGGHTNYNSALMS

SEQ ID NO: 15 - protein, 10 aa, unidentified
EVRRDWYFDV

SEQ ID NO: 16 - protein, 11 aa, unidentified
RASENIYSYLT

SEQ ID NO: 17 - protein, 7 aa, unidentified
NAKILAE

SEQ ID NO: 18 - protein, 9 aa, unidentified
QHHFGTPFT

SEQ ID NO: 19 - protein, 118 aa, unidentified
QVQLQESGPGLVKPSETLSLTCTVSGGSISNYGVHWIRQPPGKGLEWIGLIWAGGHTNYNSALMSRVTISKDNSKSQISLKLSSVTAADTAVYYCAREVRRDWYFDVWGQGTMVTVSS

SEQ ID NO: 20 - protein, 107 aa, unidentified
DIQMTQSPSSLSASVGDRVTITCRASENIYSYLTWYQQKPGKAPKLLIYNAKILAEGVPSRFSGSGSGTDFTLTISSLQPEDFATYYCQHHFGTPFTFGQGTKLEIK

SEQ ID NO: 21 - protein, 118 aa, unidentified
QVQLQESGPGLVKPSQTLSLTCAVYGGSFSNYGVHWIRQPPGKGLEWIGLIWAGGHTNYNSALMSRVTISKDNSKSQISLKLSSVTAADTAVYYCAREVRRDWYFDVWGQGTMVTVSS

SEQ ID NO: 22 - protein, 107 aa, unidentified
DIQMTQSPSTLSASVGDRVTITCRASENIYSYLTWYQQKPGKAPKLLIYNAKILAEGVPSRFSGSGSGTEFTLTISSLQPDDFATYYCQHHFGTPFTFGQGTKLEIK

SEQ ID NO: 23 - protein, 107 aa, unidentified
EIVMTQSPATLSVSPGERATLSCRASENIYSYLTWYQQKPGQAPRLLIYNAKILAEGIPARFSGSGSGTEFTLTISSLQSEDFAVYYCQHHFGTPFTFGQGTKLEIK

SEQ ID NO: 24 - protein, 5 aa, unidentified
DNYMH

SEQ ID NO: 25 - protein, 17 aa, unidentified
WIDPENGDTEYDPKFQG

SEQ ID NO: 26 - protein, 11 aa, unidentified
ITMATPYPMDY

SEQ ID NO: 27 - protein, 10 aa, unidentified
SASTSVIYMH

SEQ ID NO: 28 - protein, 7 aa, unidentified
STSNLAS

SEQ ID NO: 29 - protein, 9 aa, unidentified
QQRSSYPLT

SEQ ID NO: 30 - protein, 120 aa, unidentified
EVQLVESGGGLVQPGGSLRLSCAASGFNIKDNYMHWVRQAPGKGLEWVAWIDPENGDTEYDPKFQGRFTISADTSKNTAYLQMNSLRAEDTAVYYCSRITMATPYPMDYWGQGTLVTVSS

SEQ ID NO: 31 - protein, 107 aa, unidentified
DIQMTQSPSSLSASVGDRVTITCSASTSVIYMHWYQQKPGKAPKLLIYSTSNLASGVPSRFSGSRSGTDFTLTISSLQPEDFATYYCQQRSSYPLTFGQGTKVEIKR

SEQ ID NO: 32 - protein, 120 aa, unidentified
EVQLVESGGGLVQPGGSLRLSCAASGFNIKDNYMHWVRQAPGKGLEWVAWIDPENGDTEYDPKFQGRATMSADTSKNTAYLQMNSLRAEDTAVYYCNIITMATPYPMDYWGQGTLVTVSS

SEQ ID NO: 33 - protein, 107 aa, unidentified
DIQMTQSPSSLSASVGDRVTITCSASTSVIYMHWYQQKPGKAPKLLIYSTSNLASGVPSRFSGSGSGTDYTLTISSLQPEDFATYYCQQRSSYPLTFGQGTKVEIKR

SEQ ID NO: 34 - protein, 120 aa, unidentified
EVQLVESGGGLVQPGGSLRLSCAASGFNIKDNYMHWVRQAPGKGLEWIGWIDPENGDTEYDPKFQGRATMSADTSKNTAYLQMNSLRAEDTAVYYCNIITMATPYPMDYWGQGTLVTVSS

SEQ ID NO: 35 - protein, 107 aa, unidentified
DIQLTQSPSSLSASVGDRVTITCSASTSVIYMHWFQQKPGKAPKLWIYSTSNLASGVPSRFSGSGSGTDYTLTISSLQPEDFATYYCQQRSSYPLTFGQGTKVEIKR

SEQ ID NO: 36 - protein, 120 aa, unidentified
EVQLVQSGAEVKKPGATVKISCKVSGFNIKDNYMHWVQQAPGKGLEWIGWIDPENGDTEYDPKFQGRATMTADTSTDTAYMELSSLRSEDTAVYYCNIITMATPYPMDYWGQGTLVTVSS

SEQ ID NO: 37 - protein, 107 aa, unidentified
EIVLTQSPATLSLSPGERATLSCSASTSVIYMHWFQQKPGQAPRLWIYSTSNLASGIPARFSGSGSGTDYTLTISSLEPEDFAVYYCQQRSSYPLTFGQGTKLEIKR

SEQ ID NO: 38 - protein, 120 aa, unidentified
QVQLVQSGAEVKKPGASVKVSCKASGFNIKDNYMHWVRQAPGQGLEWIGWIDPENGDTEYDPKFQGRATMTADTSISTAYMELSRLRSDDTAVYYCNIITMATPYPMDYWGQGTLVTVSS

SEQ ID NO: 39 - protein, 107 aa, unidentified
EIVLTQSPDFQSVTPKEKVTITCSASTSVIYMHWFQQKPDQSPKLWIYSTSNLASGVPSRFSGSGSGTDYTLTINSLEAEDAATYYCQQRSSYPLTFGQGTKLEIKR

SEQ ID NO: 40 - protein, 10 aa, unidentified
GITFSRYAMS

SEQ ID NO: 41 - protein, 16 aa, unidentified
SISSDAITYYLDSVKG

SEQ ID NO: 42 - protein, 11 aa, unidentified
IYYYGSPFFDY

SEQ ID NO: 43 - protein, 11 aa, unidentified
KASQNVYTNVA

SEQ ID NO: 44 - protein, 7 aa, unidentified
SASNRYS

SEQ ID NO: 45 - protein, 10 aa, unidentified
QQYNNYPLFT

SEQ ID NO: 46 - protein, 16 aa, unidentified
SISSDAITYYLDAVKG

SEQ ID NO: 47 - protein, 668 aa, unidentified
KLTIESTPFNVAEGKEVLLLVHNLPQHLFGYSWYKGERVDGNRQIIGYVIGTQQATPGPAYSGREIIYPNASLLIQNIIQNDTGFYTLHVIKSDLVNEEATGQFRVYPELPKPSISSNNSKPVEDKDAVAFTCEPETQDATYLWWVNNQSLPVSPRLQLSNGNRTLTLFNVTRNDTASYKCETQNPVSARRSDSVILNVLYGPDAPTISPLNTSYRSGENLNLSCHAASNPPAQYSWFVNGTFQQSTQELFIPNITVNNSGSYTCQAHNSDTGLNRTTVTTITVYAEPPKPFITSNNSNPVEDEDAVALTCEPEIQNTTYLWWVNNQSLPVSPRLQLSNDNRTLTLLSVTRNDVGPYECGIQNELSVDHSDPVILNVLYGPDDPTISPSYTYYRPGVNLSLSCHAASNPPAQYSWLIDGNIQQHTQELFISNITEKNSGLYTCQANNSASGHSRTTVKTITVSAELPKPSISSNNSKPVEDKDAVAFTCEPEAQNTTYLWWVNGQSLPVSPRLQLSNGNRTLTLFNVTRNDARAYVCGIQNSVSANRSDPVTLDVLYGPDTPIISPPDSSYLSGANLNLSCHSASNPSPQYSWRINGIPQQHTQVLFIAKITPNNNGTYACFVSNLATGRNNSIVKSITVSASGTSPGLSAGATVGIMIGVLVGVALI

SEQ ID NO: 48 - protein, 189 aa, unidentified
VSAELPKPSISSNNSKPVEDKDAVAFTCEPEAQNTTYLWWVNGQSLPVSPRLQLSNGNRTLTLFNVTRNDARAYVCGIQNSVSANRSDPVTLDVLYGPDTPIISPPDSSYLSGANLNLSCHSASNPSPQYSWRINGIPQQHTQVLFIAKITPNNNGTYACFVSNLATGRNNSIVKSITVSASGTSPGLS